European Patent Specification EP 3 351 617 B1, published July 24, 2024. Title: Novel lactic acid bacteria with various functionality and use thereof. Applicant: University-Industry Cooperation Group of Kyung Hee University. The sequence listing filed with the application follows.

SEQUENCE LISTING (8 sequences)

SEQ ID NO: 1 - DNA, 1132 bp, Unknown
  16S rDNA of Lactobacillus brevis CH23
agggataacacttggaaacaggtgctaataccgtataacaacaaaatccgcatggattttgtttgaaaggtggcttcggctatcacttctggatgatcccgcggcgtattagttagttggtgaggtaaaggcccaccaagacgatgatacgtagccgacctgagagggtaatcggccacattgggactgagacacggcccaaactcctacgggaggcagcagtagggaatcttccacaatggacgaaagtctgatggagcaatgccgcgtgagtgaagaagggtttcggctcgtaaaactctgttgttaaagaagaacacctttgagagtaactgttcaagggttgacggtatttaaccagaaagccacggctaactacgtgccagcagccgcggtaatacgtaggtggcaagcgttgtccggatttattgggcgtaaagcgagcgcaggcggttttttaagtctgatgtgaaagccttcggcttaaccggagaagtgcatcggaaactgggagacttgagtgcagaagaggacagtggaactccatgtgtagcggtggaatgcgtagatatatggaagaacaccagtggcgaaggcggctgtctagtctgtaactgacgctgaggctcgaaagcatgggtagcgaacaggattagataccctgstagtccatgccgtaaacgatgagtgctaagtgttggagggtttccgcccttcagtgctgcagctaacgcattaagcactccgcctggggagtacgaccgcaaggttgaaactcaaaggaattgacgggggcccgcacaagcggtggagcatgtggtttaattcgaagctacgcgaagaaccttaccaggtcttgacatcttctgccaatcttagagataagacgttcccttcggggacagaatgacaggtggtgcatggttgtcgtcagctcgtgtcgtgagatgttgggttaagtcccgcaacgagcgcaacccttattatcagttgccagcattcagttgggcactctggtgagactgccggtgacaaaccggaggaaggtggggatgacgtcaaatcatcatgccccttatgacctgggctacacacgtgctacaatggacggtacaacgagtcgcgaagtcgt

SEQ ID NO: 2 - DNA, 1258 bp, Unknown
  16S rDNA of Lactobacillus johnsonii CH32
gtaacttgcccaagagactgggataacacctggaaacagatgctaataccggataacaacactagacgcatgtctagagtttgaaagatggttctgctatcactcttggatggacctgcggtgcattagctagttggtaaggtaacggcttaccaaggcaatgatgcatagccgagttgagagactgatcggccacattgggactgagacacggcccaaactcctacgggaggcagcagtagggaatcttccacaatggacgaaagtctgatggagcaacgccgcgtgagtgaagaagggtttcggctcgtaaagctctgttggtagtgaagaaagatagaggtagtaactggccttgatttgacggtaattccccagaaagtcacggctaactacgtgccagcagccgcggtaatacgtaggtggcaagcgttgtccggatttattgggcgtaaagcgagtgcaggcggttcaataagtctgatgtgaaagccttcggctcaaccggagaattgcatcagaaactgttgaacttgagtgcagaagaggagagtggaactccatgtgtagcggtggaatgcgtagatatatggaagaacaccagtggcgaaggcggctctctggtctgcaactgacgctgaggctcgaaagcatgggtagcgaacaggattagataccctggtagtccatgccgtaaacgatgagtgctaagtgttgggaggtttccgcctctcagtgctgcagctaacgcattaagcactccgcctggggagtacgaccgcaaggttgaaactcaaaggaattgacgggggcccgcacaagcggtggagcatgtggtttaattcgaagcaacgcgaagaaccttaccaggtcttgacatccagtgcaaacctaagagattaggtgttcccttcggggacgctgagacaggtggtgcatggctgtcgtcagctcgtgtcgtgagatgttgggttaagtcccgcaacgagcgcaacccttgtcattagttgccatcattaagttgggcactctaatgagactgccggtgacaaaccggaggaaggtggggatgacgtcaagtcatcatgccccttatgacctgggctacacacgtgctacaatggacggtacaacgagaagcgaacctgcgaaggcaagcggatctcttaaagccgttctcagttcggactgtaggctgcaactcgcctacacgaagctggaatcgctagtaatcgcggaacagtacgccgcggtgaat

SEQ ID NO: 3 - DNA, 1348 bp, Unknown
  16S rDNA of Bifidobacterium longum CH57
cgggctttgcttggtggtgagagtggcgaacgggtgagtaatgcgtgaccgacctgccccatacaccggaatagctcctggaaacgggtggtaatgccggatgctccagttgatcgcatggtcttctgggaaagctttcgcggtatgggatggggtcgcgtcctatcagcttgacggcggggtaacggcccaccgtggcttcgacgggtagccggcctgagagggcgaccggccacattgggactgagatacggcccagactcctacgggaggcagcagtggggaatattgcacaatgggcgcaagcctgatgcagcgacgccgcgtgagggatggaggccttcgggttgtaaacctcttttatcggggagcaagcgagagtgagtttacccgttgaataagcaccggctaactacgtgccagcagccgcggtaatacgtagggtgcaagcgttatccggaattattgggcgtaaagggctcgtaggcggttcgtcgcgtccggtgtgaaagtccatcgcttaacggtggatccgcgccgggtacgggcgggcttgagtgcggtaggggagactggaattcccggtgtaacggtggaatgtgtagatatcgggaagaacaccaatggcgaaggcaggtctctgggccgttactgacgctgaggagcgaaagcgtggggagcgaacaggattagataccctggtagtccacgccgtaaacggtggatgctggatgtggggcccgttccacgggttccgtgtcggagctaacgcgttaagcatcccgcctgggggagtacggccgcaaggctaaaactcaaagaaattgacgggggcccgcacaagcggcggagcatgcggattaattcgatgcaacgcgaagaaccttacctgggcttcacatgttcccgacggtcgtagagatacggcttcccttcggggcgggttcacaggtggtgcatggtcgtcgtcagctcgtgtcgtgagatgttgggttaagtcccgcaacgagcgcaaccctcgccccgtgttgccagcggattatgccgggaactcacgggggaccgccggggttaactcggaggaaggtggggatgacgtcagatcatcatgccccttacgtccagggcttcacgcatgctacaatggccggtacaacgggatgcgacgcggcgacgcggagcggatccctgaaaaccggtctcagttcggatcgcagtctgcaactcgactgcgtgaaggcggagtcgctagtaatcgcgaatcagcaacgtcgcggtgaatgcgttcccgggccttgtacacaccgcccgtcaagtcatgaaagtgggcagcacccgaagccggtgg

SEQ ID NO: 4 - DNA, 1421 bp, Unknown
  16S rDNA of Lactobacillus plantarum LC5
ctggtattgattggtgcttgcatcatgatttacatttgagtgagtggcgaactggtgagtaacacgtgggaaacctgcccagaagcgggggataacacctggaaacagatgctaataccgcataacaacttggaccgcatggtccgagcttgaaagatggcttcggctatcacttttggatggtcccgcggcgtattagctagatggtggggtaacggctcaccatggcaatgatacgtagccgacctgagagggtaatcggccacattgggactgagacacggcccaaactcctacgggaggcagcagtagggaatcttccacaatggacgaaagtctgatggagcaacgccgcgtgagtgaagaagggtttcggctcgtaaaactctgttgttaaagaagaacatatctgagagtaactgttcaggtattgacggtatttaaccagaaagccacggctaactacgtgccagcagccgcggtaatacgtaggtggcaagcgttgtccgggatttattgggcgtaaagcgagcgcaggcggttttttaagtctgatgtgaaagccttcggctcaaccgaagaagtgcatcggaaactgggaaacttgagtgcagaagaggacagtggaactccatgtgtagcggtgaaatgcgtagatatatggaagaacaccagtggcgaaggcggctgtctggtctgtaactgacgctgaggctcgaaagtatgggtagcaaacaggattagataccctggtagtccataccgtaaacgatgaatgctaagtgttggagggtttccgcccttcagtgctgcagctaacgcattaagcattccgcctggggagtacggccgcaaggctgaaactcaaaggaattgacgggggcccgcacaagcggtggagcatgtggtttaattcgaagctacgcgaagaaccttaccaggtcttgacatactatgcaaatctaagagattagacgttcccttcggggacatggatacaggtggtgcatggttgtcgtcagctcgtgtcgtgagatgttgggttaagtcccgcaacgagcgcaacccttattatcagttgccagcattaagttgggcactctggtgagactgccggtgacaaaccggaggaaggtggggatgacgtcaaatcatcatgccccttatgacctgggctacacacgtgctacaatggatggtacaacgagttgcgaactcgcgagagtaagctaatctcttaaagccattctcagttcggattgtaggctgcaactcgcctacatgaagtcggaatcgctagtaatcgcggatcagcatgccgcggtgaatacgttcccgggccttgtacacaccgcccgtcacaccatgagagtttgtaacacccaaagtcggtggggtaaccttttaggaaccagccgcct

SEQ ID NO: 5 - DNA, 1356 bp, Unknown
  16S rDNA of Lactobacillus plantarum LC27
tttacatttgattgagtggcgaactggtgagtaacacgtgggaaacctgcccagaagcgggggataacacctggaaacagatgctaataccgcataacaacttggaccgcatggtccgagtttgaaagatggcttcggctatcacttttggatggtcccgcggcgtattagctagatggtggggtaacggctcaccatggcaatgatacgtagccgacctgagagggtaatcggccacattgggactgagacacggcccaaactcctacgggaggcagcagtagggaatcttccacaatggacgaaagtctgatggagcaacgccgcgtgagtgaagaagggtttcggctcgtaaaactctgttgttaaagaagaacatatctgagagtaactgttcaggtattgacggtatttaaccagaaagccacggctaactacgtgccagcagccgcggtaatacgtaggtggcaagcgttgtccggatttattgggcgtaaagcgagcgcaggcggttttttaagtctgatgtgaaagccttcggctcaaccgaagaagtgcatcggaaactgggaaacttgagtgcagaagaggacagtggaactccatgtgtagcggtgaaatgcgtagatatatggaagaacaccagtggcgaaggcggctgtctggtctgtaactgacgctgaggctcgaaagtatgggtagcaaacaggattagataccctggtagtccataccgtaaacgatgaatgctaagtgttggagggtttccgcccttcagtgctgcagctaacgcattaagcattccgcctggggagtacggccgcaaggctgaaactcaaaggaattgacgggggcccgcacaagcggtggagcatgtggtttaattcgaagctacgcgaagaaccttaccaggtcttgacatactatgcaaatctaagagattagacgttcccttcggggacatggatacaggtggtgcatggttgtcgtcagctcgtgtcgtgagatgttgggttaagtcccgcaacgagcgcaacccttattatcagttgccagcattaagttgggcactctggtgagactgccggtgacaaaccggaggaaggtggggatgacgtcaaatcatcatgccccttatgacctgggctacacacgtgctacaatggatggtacaacgagttgcgaactcgcgagagtaagctaatctcttaaagccattctcagttcggattgtaggctgcaactcgcctacatgaagtcggaatcgctagtaatcgcggatcagcatgccgcggtgaatacgttcccgggccttgtacacaccgcccgtcacaccatgagagtttgtaacaccca

SEQ ID NO: 6 - DNA, 1325 bp, Unknown
  16S rDNA of Lactobacillus plantarum LC28
catcatgatttacatttgagtgagtggcgaactggtgagtaacacgtgggaaacctgcccagaagcgggggataacacctggaaacagatgctaataccgcataacaacttggaccgcatggtccgagtttgaaagatggcttcggctatcacttttggatggtcccgcggcgtattagctagatggtggggtaacggctcaccatggcaatgatacgtagccgacctgagagggtaatcggccacattgggactgagacacggcccaaactcctacgggaggcagcagtagggaatcttccacaatggacgaaagtctgatggagcaacgccgcgtgagtgaagaagggtttcggctcgtaaaactctgttgttaaagaagaacatatctgagagtaactgttcaggtattgacggtatttaaccagaaagccacggctaactacgtgccagcagccgcggtaatacgtaggtggcaagcgttgtccggatttattgggcgtaaagcgagcgcaggcggttttttaagtctgatgtgaaagccttcggctcaaccgaagaagtgcatcggaaactgggaaacttgagtgcagaagaggacagtggaactccatgtgtagcggtgaaatgcgtagatatatggaagaacaccagtggcgaaggcggctgtctggtctgtaactgacgctgaggctcgaaagtatgggtagcaaacaggattagataccctggtagtccataccgtaaacgatgaatgctaagtgttggagggtttccgcccttcagtgctgcagctaacgcattaagcattccgcctggggagtacggccgcaaggctgaaactcaaaggaattgacgggggcccgcacaagcggtggagcatgtggtttaattcgaagctacgcgaagaaccttaccaggtcttgacatactatgcaaatctaagagattagacgttcccttcggggacatggatacaggtggtgcatggttgtcgtcagctcgtgtcgtgagatgttgggttaagtcccgcaacgagcgcaacccttattatcagttgccagcattaagttgggcactctggtgagactgccggtgacaaaccggaggaaggtggggatgacgtcaaatcatcatgccccttatgacctgggctacacacgtgctacaatggatggtacaacgagttgcgaactcgcgagagtaagctaatctcttaaagccattctcagttcggattgtaggctgcaactcgcctacatgaagtcggaatcgctagtaatcgcggatcagcattccgcggtgaatacgttcccgggccttgt

SEQ ID NO: 7 - DNA, 1342 bp, Unknown
  16S rDNA of Bifidobacterium longum LC67
ggctttgcttggtggtgagagtggcgaacgggtgagtaatgcgtgaccgacctgccccatacaccggaatagctcctggaaacgggtggtaatgccggatgctccagttgatcgcatggtcttctgggaaagctttcgcggtatgggatggggtcgcgtcctatcagcttgacggcggggtaacggcccaccgtggcttcgacgggtagccggcctgagagggcgaccggccacattgggactgagatacggcccagactcctacgggaggcagcagtggggaatattgcacaatgggcgcaagcctgatgcagcgacgccgcgtgagggatggaggccttcgggttgtaaacctcttttatcggggagcaagcgagagtgagtttacccgttgaataagcaccggctaactacgtgccagcagccgcggtaatacgtagggtgcaagcgttatcccggaattattgggcgtaaagggctcgtaggcggttcgtcgcgtccggtgtgaaagtccatcgcttaacggtggatccgcgccgggtacgggcgggcttgagtgcggtaggggagactggaattcccggtgtaacggtggaatgtgtagatatcgggaagaacaccaatggcgaaggcaggtctctgggccgttactgacgctgaggagcgaaagcgtggggagcgaacaggattagataccctggtagtccacgccgtaaacggtggatgctggatgtggggcccgttccacgggttccgtgtcggagctaacgcgttaagcatcccgcctgggggagtacggccgcaaggctaaaactcaaagaaattgacgggggcccgcacaagcggcggagcatgcggattaattcgatgcaacgcgaagaaccttacctgggcttgacatgttcccgacggtcgtagagatacggcttcccttcggggcgggttcacaggtggtgcatggtcgtcgtcagctcgtgtcgtgagatgttgggttaagtcccgcaacgagcgcaaccctcgccccgtgttgccagcggattatgccgggaactcacgggggaccgccggggttaactcggaggaaggtggggatgacgtcagatcatcatgccccttacgtccagggcttcacgcatgctacaatggccggtacaacgggatgcgacgcggcgacgcggagcggatccctgaaaaccggtctcagttcggatcgcagtctgcaactcgactgcgtgaaggcggagtcgctagtaatcgcgaatcagcaacgtcgcggtgaatgcgttcccgggccttgtacacaccgcccgtcaagtcatgaaagtgggcagcacccgaagcg

SEQ ID NO: 8 - DNA, 1343 bp, Unknown
  16S rDNA of Bifidobacterium longum LC68
cggcttcgggtgctgcccactttcatgacttgacgggcggtgtgtacaaggcccgggaacgcattcaccgcgacgttgctgattcgcgattactagcgactccgccttcacgcagtcgagttgcagactgcgatccgaactgagaccggttttcagggatccgctccgcgtcgccgcgtcgcatcccgttgtaccggccattgtagcatgcgtgaagccctggacgtaaggggcatgatgatctgacgtcatccccaccttcctccgagttaaccccggcggtcccccgtgagttcccggcataatccgctggcaacacggggcgagggttgcgctcgttgcgggacttaacccaacatctcacgacacgagctgacgacgaccatgcaccacctgtgaacccgccccgaagggaagccgcatctctacgaccgtcgggaacatgtcaagcccaggtaaggttcttcgcgttgcatcgaattaatccgcatgctccgccgcttgtgcgggcccccgtcaatttctttgagttttagccttgcggccgtactccccaggcgggatgcttaacgcgttagctccgacacggaacccgtggaacgggccccacatccagcatccaccgtttacggcgtggactaccagggtatctaatcctgttcgctccccacgctttcgctcctcagcgtcagtaacggcccagagacctgccttcgccattggtgttcttcccgatatctacacattccaccgttacaccgggaattccagtctcccctaccgcactcaagcccgcccgtacccggcgcggatccaccgttaagcgatggactttcacaccggacgcgacgaaccgcctacgagccctttacgcccaataattccggataacgcttgcaccctacgtattaccgcggctgctggcacgtagttagccggtgcttattcaacgggtaaactcactctcgcttgctccccgataaaagaggtttacaacccgaaggcctccatccctcacgcggcgtcgctgcatcaggcttgcgcccattgtgcaatattccccactgctgcctcccgtaggagtctgggccgtatctcagtcccaatgtggccggtcgccctctcaggccggctacccgtcgaagccacggtgggccgttaccccgccgtcaagctgataggacgcgaccccatcccataccgcgaaagctttcccagaagaccatgcgatcaactggagcatccggcattaccacccgtttccaggagctattccggtgtatggggcaggtcggtcacgcattactcacccgttcgccactctcaccaccaagcaaagtctc